European Patent Specification EP 3 399 021 B1, published March 15, 2023. Title: OMV VACCINES. Applicant: NOVARTIS AG. Application PCT/IB2011/002341. The sequence listing filed with the application follows.

SEQUENCE LISTING (86 sequences)

SEQ ID NO: 1 - protein, 497 aa, Chlamydia trachomatis
MMKRLLCVLLSTSVFSSPMLGYSASKKDSKADICLAVSSGDQEVSQEDLLKEVSRGFSRVAAKATPGVVYIENFPKTGNQAIASPGNKRGFQENPFDYFNDEFFNRFFGLPSHREQQRPQQRDAVRGTGFIVSEDGYVVTNHHVVEDAGKIHVTLHDGQKYTAKIVGLDPKTDLAVIKIQAEKLPFLTFGNSDQLQIGDWAIAIGNPFGLQATVTVGVISAKGRNQLHIVDFEDFIQTDAAINPGNSGGPLLNINGQVIGVNTAIVSGSGGYIGIGFAIPSLMAKRVIDQLISDGQVTRGFLGVTLQPIDSELATCYKLEKVYGALVTDVVKGSPAEKAGLRQEDVIVAYNGKEVESLSALRNAISLMMPGTRVVLKIVREGKTIEIPVTVTQIPTEDGVSALQKMGVRVQNITPEICKKLGLAADTRGILVVAVEAGSPAASAGVAPGQLILAVNRQRVASVEELNQVLKNSKGENVLLMVSQGDVVRFIVLKSDE

SEQ ID NO: 2 - DNA, 1494 bp, Chlamydia trachomatis
atgatgaaaagattattatgtgtgttgctatcgacatcagttttctcttcgccaatgctaggctatagtgcgtcaaagaaagattctaaggctgatatttgtcttgcagtatcctcaggagatcaagaggtttcacaagaagatctgctcaaagaagtatcccgaggattttctcgggtcgctgctaaggcaacgcctggagttgtatatatagaaaattttcctaaaacagggaaccaggctattgcttctccaggaaacaaaagaggctttcaagagaacccttttgattattttaatgacgaattttttaatcgattttttggattgccttcgcatagagagcagcagcgtccgcagcagcgtgatgctgtaagaggaactgggttcattgtttctgaagatggttatgttgttactaaccatcatgtagtcgaggatgcaggaaaaattcatgttactctccacgacggacaaaaatacacagctaagatcgtggggttagatccaaaaacagatcttgctgtgatcaaaattcaagcggagaaattaccatttttgacttttgggaattctgatcagctgcagataggtgactgggctattgctattggaaatccttttggattgcaagcaacggtcactgtcggggtcattagtgctaaaggaagaaatcagctacatattgtagatttcgaagactttattcaaacagatgctgccattaatcctgggaattcaggcggtccattgttaaacatcaatggtcaagttatcggggttaatactgccattgtcagtggtagcgggggatatattggaatagggtttgctattcctagcttgatggctaaacgagtcattgatcaattgattagtgatgggcaggtaacaagaggctttttgggagttaccttgcaaccgatagattctgaattggctacttgttacaaattggaaaaagtgtacggagctttggtgacggatgttgttaaaggttctccagcagaaaaagcagggctgcgccaagaagatgtcattgtggcttacaatggaaaagaagtagagtctttgagtgcgttgcgtaatgccatttccctaatgatgccagggactcgtgttgttttaaaaatcgttcgtgaagggaaaacaatcgagatacctgtgacggttacacagatcccaacagaggatggcgtttcagcgttgcagaagatgggagtccgtgttcagaacattactccagaaatttgtaagaaactcggattggcagcagatacccgagggattctggtagttgctgtggaggcaggctcgcctgcagcttctgcaggcgtcgctcctggacagcttatcttagcggtgaataggcagcgagtcgcttccgttgaagagttaaatcaggttttgaaaaactcgaaaggagagaatgttctccttatggtttctcaaggagatgtggtgcgattcatcgtcttgaaatcagacgagtag

SEQ ID NO: 3 - DNA, 1347 bp, Chlamydia trachomatis
atgttaataaactttacctttcgcaactgtcttttgttccttgtcacactgtctagtgtccctgttttctcagcacctcaacctcgcggaacgcttcctagctcgaccacaaaaattggatcagaagtttggattgaacaaaaagtccgccaatatccagagcttttatggttagtagagccgtcctctacgggagcctctttaaaatctccttcaggagccatcttttctccaacattattccaaaaaaaggtccctgctttcgatatcgcagtgcgcagtttgattcacttacatttattaatccagggttcccgccaagcctatgctcaactgatccaactacagaccagcgaatcccctctaacatttaagcaattccttgcattgcataagcaattaactctatttttaaattcccctaaggaattttatgactctgttaaagtgttagagacagctatcgtcttacgtcacttaggctgttcaactaaggctgttgctgcgtttaaaccttatttctcagaaatgcaaagagaggctttttacactaaggctctgcatgtactacacaccttcccagagctaagcccatcatttgctcgcctctctccggagcagaaaactctcttcttctccttgagaaaattggcgaattacgatgagttactctcgctgacgaacaccccaagttttcagcttctgtctgctgggcgctcgcaacgagctcttttagctctggacttgtacctctatgctttggattcctgtggagaacaggggatgtcctctcaattccacacaaacttcgcacctctacagtccatgttgcaacaatacgctactgtagaagaggccttttctcgttattttacttaccgagctaatcgattaggatttgatggctcttctcgatccgagatggctttagtaagaatggccaccttgatgaacttgtctccttccgaagctgcgattttaaccacaagcttcaaaacccttcctacagaagaagcggatactttgatcaatagtttctataccaataagggcgattcgttggctctttctctgcgagggttgcctacacttgtatccgaactgacgcgaactgcccatggcaataccaatgcagaagctcgatctcagcaaatttatgcaactaccctatcgctagtagtaaagagtctgaaagcgcacaaagaaatgctaaacaagcaaattctttctaaggaaattgttttagatttctcagaaactgcagcttcttgccaaggattggatatcttttccgagaatgtcgctgttcaaattcacttaaatggaaccgttagtatccatttataa

SEQ ID NO: 4 - protein, 448 aa, Chlamydia trachomatis
MLINFTFRNCLLFLVTLSSVPVFSAPQPRGTLPSSTTKIGSEVWIEQKVRQYPELLWLVEPSSTGASLKSPSGAIFSPTLFQKKVPAFDIAVRSLIHLHLLIQGSRQAYAQLIQLQTSESPLTFKQFLALHKQLTLFLNSPKEFYDSVKVLETAIVLRHLGCSTKAVAAFKPYFSEMQREAFYTKALHVLHTFPELSPSFARLSPEQKTLFFSLRKLANYDELLSLTNTPSFQLLSAGRSQRALLALDLYLYALDSCGEQGMSSQFHTNFAPLQSMLQQYATVEEAFSRYFTYRANRLGFDGSSRSEMALVRMATLMNLSPSEAAILTTSFKTLPTEEADTLINSFYTNKGDSLALSLRGLPTLVSELTRTAHGNTNAEARSQQIYATTLSLVVKSLKAHKEMLNKQILSKEIVLDFSETAASCQGLDIFSENVAVQIHLNGTVSIHL

SEQ ID NO: 5 - DNA, 2433 bp, Chlamydia trachomatis
atgactaagccttctttcttatacgttattcaacctttttccgtatttaatccacgattaggacgtttctctacagactcagatacttatatcgaagaagaaaaccgcctagcatcgttcattgagagtttgccactggagatcttcgatataccttctttcatggaaaccgcgatttccaatagcccctatattttatcttgggagacaactaaagacggcgctctgttcactattcttgaacccaaactctcagcttgcgcagccacttgcctggtagccccttctatacaaatgaaatccgatgcggagctcctagaagaaattaagcaagcgttattacgcagctctcatgacggtgtgaaatatcgcatcaccagagaatccttctctccagaaaagaaaactcctaaggttgctctagtcgatgacgatattgaattgattcgcaatgtcgactttttgggtagagctgttgacattgtcaaattagaccctattaatattctgaataccgtaagcgaagagaatattctagattactcttttacaagagaaacggctcagctgagcgcggatggtcgttttggtattcctccagggactaagctattccctaaaccttcttttgatgtagaaatcagtacctccattttcgaagaaacaacttcatttactcgaagtttttctgcatcggttacttttagtgtaccagacctcgcggcgactatgcctcttcaaagccctcccatggtagaaaatggtcaaaaagaaatttgtgtcattcaaaaacacttattcccaagctactctcctaaactagtcgatattgttaaacgatacaaaagagaggctaagatcttgattaacaagcttgcctttggaatgttatggcgacatcgggctaaaagccaaatcctcaccgagggaagcgtacgtctagacttacaaggattcacagaatcgaagtacaattaccagattcaagtaggatcccatacgattgcagctgtattaatcgatatggatatttccaagattcaatccaaatcagaacaagcttatgcaattaggaaaatcaaatcaggctttcaacgtagcttggatgactatcatatttatcaaattgaaagaaaacaaaccttttctttttctccgaagcatcgcagcctctcatccacatcccattccgaagattctgatttggatctttctgaagcagccgccttttcaggaagtcttacctgcgagtttgtaaaaaaaagcactcaacatgccaagaataccgtcacatgttccacagccgctcattccctatacacactcaaagaagatgacagctcgaacccctctgaaaaacgattagatagttgtttccgcaattggattgaaaacaaactaagcgccaattctccagattcctggtcagcgtttattcaaaaattcggaacacactatattgcatcagcaacttttggagggataggtttccaagtgctcaaactatcttttgaacaggtggaggatctacatagcaaaaagatctccttagaaaccgcagcagccaactctctattaaaaggttctgtatccagcagcacagaatctggatactccagctatagctccacgtcttcttctcatacggtatttttaggaggaacggtcttaccttcggttcatgatgaacgtttagactttaaagattggtcggaaagtgtgcacctggaacctgttcctatccaggtttctttacaacctataacgaatttactagttcctctccattttcctaatatcggtgctgcagagctctctaataaacgagaatctcttcaacaagcgattcgagtctatctcaaagaacataaagtagatgagcaaggagaacgtactacatttacatcaggaatcgataatccttcttcctggtttaccttagaagctgcccactctcctcttatagtcagtactccttacattgcttcgtggtctacgcttccttatttgttcccaacattaagagaacgttcttcggcaacccctatcgttttctatttttgtgtagataataatgaacatgcttcgcaaaaaatattaaaccaatcgtattgcttcctcgggtccttgcctattcgacaaaaaatttttggtagcgaatttgctagtttcccctatctatctttctatggaaatgcaaaagaggcgtactttgataacacgtactacccaacgcgttgtgggtggattgttgaaaagttaaatactacacaagatcaattcctccgggatggagacgaggtgcgactaaaacatgtttccagcggaaagtatctagcaacaactcctcttaaggatacccatggtacactcacgcgtacaacgaactgtgaagatgctatctttattattaaaaaatcttcaggttattga

SEQ ID NO: 6 - protein, 350 aa, Chlamydia trachomatis
MTKPSFLYVIQPFSVFNPRLGRFSTDSDTYIEEENRLASFIESLPLEIFDIPSFMETAISNSPYILSWETTKDGALFTILEPKLSACAATCLVAPSIQMKSDAELLEEIKQALLRSSHDGVKYRITRESFSPEKKTPKVALVDDDIELIRNVDFLGRAVDIVKLDPINILNTVSEENILDYSFTRETAQLSADGRFGIPPGTKLFPKPSFDVEISTSIFEETTSFTRSFSASVTFSVPDLAATMPLQSPPMVENGQKEICVIQKHLFPSYSPKLVDIVKRYKREAKILINKLAFGMLWRHRAKSQILTEGSVRLDLQGFTESKYNYQIQVGSHTIAAVLIDMDISKIQSK

SEQ ID NO: 7 - DNA, 603 bp, Chlamydia trachomatis
atgctcgctaatcgcttattcttaataacccttttagggttaagttcgtctgtttacggcgcaggtaaagcaccgtctttgcaggctattctagccgaagtcgaagacacctcctctcgtctacacgctcatcacaatgagcttgctatgatctctgaacgcctcgatgagcaagacacgaaactacagcaactttcgtcaacacaagatcataacctacctcgacaagttcagcgactagaaacggaccaaaaagctttggcaaaaacactggcgattctttcgcaatccgtccaagatattcggtcttctgtacaaaataaattacaagaaatccaacaagaacaaaaaaaattagcacaaaatttgcgagcgcttcgtaactctttacaagctctcgttgatggctcttctccagaaaattatattgatttcctaactggtgaaaccccggaacatattcatattgttaaacaaggagagaccctgagcaagatcgcgagtaaatataacatccccgtcgtagaattaaaaaaacttaataaactaaattcggatactatttttacagatcaaagaattcgccttccgaaaaagaaatag

SEQ ID NO: 8 - protein, 200 aa, Chlamydia trachomatis
MLANRLFLITLLGLSSSVYGAGKAPSLQAILAEVEDTSSRLHAHHNELAMISERLDEQDTKLQQLSSTQDHNLPRQVQRLETDQKALAKTLAILSQSVQDIRSSVQNKLQEIQQEQKKLAQNLRALRNSLQALVDGSSPENYIDFLTGETPEHIHIVKQGETLSKIASKYNIPVVELKKLNKLNSDTIFTDQRIRLPKKK

SEQ ID NO: 9 - DNA, 951 bp, Chlamydia trachomatis
atggcatccaagtctcgccattatcttaatcagccttggtacattatcttattcatctttgttcttagtttaattgctggtaccctcctgtcttctgtgtattatgtccttgcacctatccaacagcaagctgcggaattcgatcgcaatcaacaaatgctaatggctgcacaagtaatttcttccgataacacattccaagtctatgaaaagggagattggcacccagccctatataatactaaaaagcagttgctagagatctcctctactcctcctaaagtaaccgtgacaactttaagctcatattttcaaaactttgttagagtcttgcttacagatacacaaggaaatctttcttcattcgaagaccataatctcaatctagaagaatttttatctcaaccaactcctgtaatacatggtcttgccctttatgtggtctacgctatcctacacaacgatgcagcttcctctaaattatctgcttcccaagtagcgaaaaatccaacagctatagaatctatagttcttcctatagaaggttttggtttgtggggacctatctatggattccttgctctagaaaaagacgggaatactgttcttggtacttcttggtatcaacatggcgagactcctggattaggagcaaatatcgctaaccctcaatggcaaaaaaatttcagaggcaaaaaagtatttctagtctcagcttctggagaaacagattttgctaagacaaccctaggactggaagttataaaaggatctgtatctgcagcattaggagactcacctaaagctgcttcttccatcgacggaatttcaggagctactttgacttgtaatggtgttaccgaatccttctctcattctctagctccctaccgcgctttgttgactttcttcgccaactctaaacctagtggagagtctcatgaccactaa

SEQ ID NO: 10 - protein, 316 aa, Chlamydia trachomatis
MASKSRHYLNQPWYIILFIFVLSLIAGTLLSSVYYVLAPIQQQAAEFDRNQQMLMAAQVISSDNTFQVYEKGDWHPALYNTKKQLLEISSTPPKVTVTTLSSYFQNFVRVLLTDTQGNLSSFEDHNLNLEEFLSQPTPVIHGLALYVVYAILHNDAASSKLSASQVAKNPTAIESIVLPIEGFGLWGPIYGFLALEKDGNTVLGTSWYQHGETPGLGANIANPQWQKNFRGKKVFLVSASGETDFAKTTLGLEVIKGSVSAALGDSPKAASSIDGISGATLTCNGVTESFSHSLAPYRALLTFFANSKPSGESHDH

SEQ ID NO: 11 - DNA, 1662 bp, Chlamydia trachomatis
atgcgaataggagatcctatgaacaaactcatcagacgagcagtgacgatcttcgcggtgactagtgtggcgagtttatttgctagcggggtgttagagacctctatggcagagtctctctctacaaacgttattagcttagctgacaccaaagcgaaagacaacacttctcataaaagcaaaaaagcaagaaaaaaccacagcaaagagactcccgtagaccgtaaagaggttgctccggttcatgagtctaaagctacaggacctaaacaggattcttgctttggcagaatgtatacagtcaaagttaatgatgatcgcaatgttgaaatcacacaagctgttcctgaatatgctacggtaggatctccctatcctattgaaattactgctacaggtaaaagggattgtgttgatgttatcattactcagcaattaccatgtgaagcagagttcgtacgcagtgatccagcgacaactcctactgctgatggtaagctagtttggaaaattgaccgcttaggacaaggcgaaaagagtaaaattactgtatgggtaaaacctcttaaagaaggttgctgctttacagctgcaacagtatgcgcttgtccagagatccgttcggttacaaaatgtggacaacctgctatctgtgttaaacaagaaggcccagagaatgcttgtttgcgttgcccagtagtttacaaaattaatatagtgaaccaaggaacagcaacagctcgtaacgttgttgttgaaaatcctgttccagatggttacgctcattcttctggacagcgtgtactgacgtttactcttggagatatgcaacctggagagcacagaacaattactgtagagttttgtccgcttaaacgtggtcgtgctaccaatatagcaacggtttcttactgtggaggacataaaaatacagcaagcgtaacaactgtgatcaacgagccttgcgtacaagtaagtattgcaggagcagattggtcttatgtttgtaagcctgtagaatatgtgatctccgtttccaatcctggagatcttgtgttgcgagatgtcgtcgttgaagacactctttctcccggagtcacagttcttgaagctgcaggagctcaaatttcttgtaataaagtagtttggactgtgaaagaactgaatcctggagagtctctacagtataaagttctagtaagagcacaaactcctggacaattcacaaataatgttgttgtgaagagctgctctgactgtggtacttgtacttcttgcgcagaagcgacaacttactggaaaggagttgctgctactcatatgtgcgtagtagatacttgtgaccctgtttgtgtaggagaaaatactgtttaccgtatttgtgtcaccaacagaggttctgcagaagatacaaatgtttctttaatgcttaaattctctaaagaactgcaacctgtatccttctctggaccaactaaaggaacgattacaggcaatacagtagtattcgattcgttacctagattaggttctaaagaaactgtagagttttctgtaacattgaaagcagtatcagctggagatgctcgtggggaagcgattctttcttccgatacattgactgttccagtttctgatacagagaatacacacatctattaa

SEQ ID NO: 12 - protein, 553 aa, Chlamydia trachomatis
MRIGDPMNKLIRRAVTIFAVTSVASLFASGVLETSMAESLSTNVISLADTKAKDNTSHKSKKARKNHSKETPVDRKEVAPVHESKATGPKQDSCFGRMYTVKVNDDRNVEITQAVPEYATVGSPYPIEITATGKRDCVDVIITQQLPCEAEFVRSDPATTPTADGKLVWKIDRLGQGEKSKITVWVKPLKEGCCFTAATVCACPEIRSVTKCGQPAICVKQEGPENACLRCPVVYKINIVNQGTATARNVVVENPVPDGYAHSSGQRVLTFTLGDMQPGEHRTITVEFCPLKRGRATNIATVSYCGGHKNTASVTTVINEPCVQVSIAGADWSYVCKPVEYVISVSNPGDLVLRDVVVEDTLSPGVTVLEAAGAQISCNKVVWTVKELNPGESLQYKVLVRAQTPGQFTNNVVVKSCSDCGTCTSCAEATTYWKGVAATHMCVVDTCDPVCVGENTVYRICVTNRGSAEDTNVSLMLKFSKELQPVSFSGPTKGTITGNTVVFDSLPRLGSKETVEFSVTLKAVSAGDARGEAILSSDTLTVPVSDTENTHIY

SEQ ID NO: 13 - DNA, 1329 bp, Chlamydia trachomatis
atgcaggctgcacaccatcactatcaccgctacacagataaactgcacagacaaaaccataaaaaagatctcatctctcccaaacctaccgaacaagaggcgtgcaatacttcttcccttagtaaggaattaatccctctatcagaacaaagaggccttttatcccccatctgtgactttatttcggaacgcccttgcttacacggagtttctgttagaaatctcaagcaagcgctaaaaaattctgcaggaacccaaattgcactggattggtctattctccctcaatggttcaatcctcgggtctctcatgcccctaagctttctatccgagactttgggtatagcgcacaccaaactgttaccgaagccactcctccttgctggcaaaactgctttaatccatctgcggccgttactatctatgattcctcatatgggaaaggggtctttcaaatatcctatacccttgtccgctattggagagagaatgctgcgactgctggcgatgctatgatgctcgcagggagtatcaatgattatccctctcgtcagaacattttctctcagtttactttctcccaaaacttcccaaatgaacgggtgagtctgacaattggtcagtactcactctatgcaatagacggaacattatacaataacgatcaacaacttggattcattagttacgcattatcacaaaatccaacagcaacttattcctctggaagtcttggagcttacctacaagtcgctcctaccgcaagcacaagtcttcaaataggatttcaagacgcttataatatctccggatcctctatcaaatggagtaaccttacaaaaaatagatacaattttcacggttttgcttcctgggctccccgctgttgcttaggatctggccagtactccgtgcttctttatgtgactagacaagttccagaacagatggaacaaacaatgggatggtcagtcaatgcgagtcaacacatatcttctaaactgtatgtgtttggaagatacagcggtgttacaggacatgtgttcccgattaaccgcacgtattcattcggtatggcctctgcaaatttatttaaccgtaacccacaagatttatttggaattgcttgcgcattcaataatgtacacctctctgcttctccaaatactaaaagaaaatacgaaactgtaatcgaagggtttgcaactatcggttgcggcccctatctttctttcgctccagacttccaactctacctctacccagctcttcgtccaaacaaacaatctgcccgtgtttatagcgtgcgagctaatttagctatctaa

SEQ ID NO: 14 - protein, 47 aa, Chlamydia trachomatis
MQAAHHHYHRYTDKLHRQNHKKDLISPKPTEQEACNTSSLSKELIPL

SEQ ID NO: 15 - DNA, 504 bp, Chlamydia trachomatis
atgtccaggcagaatgctgaggaaaatctaaaaaattttgctaaagagcttaaactccccgacgtggccttcgatcagaataatacgtgcattttgtttgttgatggagagttttctcttcacctgacctacgaagaacactctgatcgcctttatgtttacgcacctcttcttgacggactgccagacaatccgcaaagaaggttagctctatatgagaagttgttagaaggctctatgctcggaggccaaatggctggtggaggggtaggagtcgctactaaggaacagttgatcttaatgcactgcgtgttagacatgaagtatgcagagaccaacctactcaaagcttttgcacagctttttattgaaaccgttgtgaaatggcgaactgtttgttctgatatcagcgctggacgagaacccactgttgataccatgccacaaatgcctcaagggggtggcggaggaattcaacctcctccagcaggaatccgtgcataa

SEQ ID NO: 16 - protein, 167 aa, Chlamydia trachomatis
MSRQNAEENLKNFAKELKLPDVAFDQNNTCILFVDGEFSLHLTYEEHSDRLYVYAPLLDGLPDNPQRRLALYEKLLEGSMLGGQMAGGGVGVATKEQLILMHCVLDMKYAETNLLKAFAQLFIETVVKWRTVCSDISAGREPTVDTMPQMPQGGGGGIQPPPAGIRA

SEQ ID NO: 17 - protein, 393 aa, Chlamydia trachomatis
MKKLLKSVLVFAALSSASSLQALPVGNPAEPSLMIDGILWEGFGGDPCDPCATWCDAISMRVGYYGDFVFDRVLKTDVNKEFQMGAKPTTDTGNSAAPSTLTARENPAYGRHMQDAEMFTNAACMALNIWDRFDVFCTLGATSGYLKGNSASFNLVGLFGDNENQKTVKAESVPNMSFDQSVVELYTDTTFAWSVGARAALWECGCATLGASFQYAQSKPKVEELNVLCNAAEFTINKPKGYVGKEFPLDLTAGTDAATGTKDASIDYHEWQASLALSYRLNMFTPYIGVKWSRASFDADTIRIAQPKSATAIFDTTTLNPTIAGAGDVKTGAEGQLGDTMQIVSLQLNKMKSRKSCGIAVGTTIVDADKYAVTVETRLIDERAAHVNAQFRF

SEQ ID NO: 18 - DNA, 1154 bp, Chlamydia trachomatis
atgaaaaaactcttgaaatcggtattagtatttgccgctttgagttctgcttcctccttgcaagctctgcctgtggggaatcctgctgaaccaagccttatgatcgacggaattctgtgggaaggtttcggcggagatccttgcgatccttgcgccacttggtgtgacgctatcagcatgcgtgttggttactacggagactttgttttcgaccgtgttttgaaaacagatgtgaataaagaatttcagatgggtgccaagcctacaactgatacaggcaatagtgcagctccatccactcttacagcaagagagaatcctgcttacggccgacatatgcaggatgctgagatgtttacaaatgccgcttgcatggcattgaatatttgggatcgttttgatgtattctgtacattaggagccaccagtggatatcttaaaggaaactctgcttctttcaatttagttggattgtttggagataatgaaaatcaaaaaacggtcaaagcggagtctgtaccaaatatgagctttgatcaatctgttgttgagttgtatacagatactacttttgcgtggagcgtcggcgctcgcgcagctttgtgggaatgtggatgtgcaactttaggagcttcattccaatatgctcaatctaaacctaaagtagaagaattaaacgttctctgcaatgcagcagagtttactattaataaacctaaagggtatgtaggtaaggagtttcctcttgatcttacagcaggaacagatgctgcgacaggaactaaggatgcctctattgattaccatgaatggcaagcaagtttagctctctcttacagactgaatatgttcactccctacattggagttaaatggtctcgagcaagctttgatgccgatacgattcgtatagcccagccaaaatcagctacagctatttttgatactaccacgcttaacccaactattgctggagctggcgatgtgaaaactggcgcagagggtcagctcggagacacaatgcaaatcgtttccttgcaattgaacaagatgaaatctagaaaatcttgcggtattgcagtaggaacaactattgtggatgcagacaaatacgcagttacagttgagactcgcttgatcgatgagagagcagc

SEQ ID NO: 19 - protein, 497 aa, Chlamydia muridarum
MMKRLLCVLLSTSVFSSPMLGYSAPKKDSSTGICLAASQSDRELSQEDLLKEVSRGFSKVAAQATPGVVYIENFPKTGSQAIASPGNKRGFQENPFDYFNDEFFNRFFGLPSHREQPRPQQRDAVRGTGFIVSEDGYVVTNHHVVEDAGKIHVTLHDGQKYTAKIIGLDPKTDLAVIKIQAKNLPFLTFGNSDQLQIGDWSIAIGNPFGLQATVTVGVISAKGRNQLHIVDFEDFIQTDAAINPGNSGGPLLNIDGQVIGVNTAIVSGSGGYIGIGFAIPSLMAKRVIDQLISDGQVTRGFLGVTLQPIDSELAACYKLEKVYGALITDVVKGSPAEKAGLRQEDVIVAYNGKEVESLSALRNAISLMMPGTRVVLKVVREGKFIEIPVTVTQIPAEDGVSALQKMGVRVQNLTPEICKKLGLASDTRGIFVVSVEAGSPAASAGVVPGQLILAVNRQRVSSVEELNQVLKNAKGENVLLMVSQGEVIRFVVLKSDE

SEQ ID NO: 20 - protein, 387 aa, Chlamydia muridarum
MKKLLKSVLAFAVLGSASSLHALPVGNPAEPSLMIDGILWEGFGGDPCDPCTTWCDAISLRLGYYGDFVFDRVLKTDVNKQFEMGAAPTGDADLTTAPTPASRENPAYGKHMQDAEMFTNAAYMALNIWDRFDVFCTLGATSGYLKGNSAAFNLVGLFGRDETAVAADDIPNVSLSQAVVELYTDTAFAWSVGARAALWECGCATLGASFQYAQSKPKVEELNVLCNAAEFTINKPKGYVGQEFPLNIKAGTVSATDTKDASIDYHEWQASLALSYRLNMFTPYIGVKWSRASFDADTIRIAQPKLETSILKMTTWNPTISGSGIDVDTKITDTLQIVSLQLNKMKSRKSCGLAIGTTIVDADKYAVTVETRLIDERAAHVNAQFRF

SEQ ID NO: 21 - DNA, 1164 bp, Chlamydia muridarum
atgaaaaaactcttgaaatcggtattagcatttgccgttttgggttctgcttcctccttgcatgctctgcctgtggggaatcctgctgaaccaagccttatgattgacgggattctttgggaaggtttcggtggagatccttgcgatccttgcacaacttggtgtgatgccatcagcctacgtctcggctactatggggacttcgtttttgatcgtgttttgaaaacagacgtgaacaaacagttcgaaatgggagcagctcctacaggagatgcagaccttactacagcacctactcctgcatcaagagagaatcccgcttatggcaagcatatgcaagatgcagaaatgttcactaatgctgcgtacatggctttaaacatttgggaccgtttcgatgtattttgtacattgggagcaactagcggatatcttaaaggtaattctgccgcctttaacttagttggtctgtttggaagagatgaaactgcagttgcagctgacgacatacctaacgtcagcttgtctcaagctgttgtcgaactctacacagacacagctttcgcttggagcgtcggtgctagagcagctttatgggagtgcggatgtgcaactttaggagcttccttccaatatgctcaatctaagccaaaagtagaggaattaaacgttctctgtaatgcggcagaattcactattaacaagcctaaaggatacgttggacaagagtttcctcttaacattaaagctggaacagttagcgctacagatactaaagatgcttccatcgattaccatgagtggcaagcaagcttggctttgtcttacagactgaatatgttcactccttacattggagttaagtggtctagagcaagctttgatgccgacactatccgcattgcgcagcctaagcttgagacctctatcttaaaaatgaccacttggaacccaacgatctctggatctggtatagacgttgatacaaaaatcacggatacattacaaattgtttccttgcagctcaacaagatgaaatccagaaaatcttgcggtcttgcaattggaacaacaattgtagatgctgataaatatgcagttactgttgagacacgcttgatcgatgaaagagcagctcacgtaaatgctcagttccgtttctaa

SEQ ID NO: 22 - protein, 448 aa, Chlamydia muridarum
MLTNFTFRNCLLFFVTLSSVPVFSAPQPRVTLPSGANKIGSEAWIEQKVRQYPELLWLVEPSPAGTSLNAPSGMIFSPLLFQKKVPAFDIAVRSLIHLHLLIQGSRQAYAQLVQLQANESPMTFKQFLTLHKQLSLFLNSPKEFYDSVKILETAIILRHLGCSTKAVATFKPYFSETQKEVFYTKALHVLHTFPELSPSFARLSPEQKTLFFSLRKLANYDELLSLTNAPSLQLLSAVRSRRALLALDLYLYALDFCGEQGISSQFHMDFSPLQSMLQQYATVEEAFSRYFTYRANRLGFAGSSRTEMALVRIATLMNLSPSEAAILTTSFKSLSLEDAESLVNSFYTNKGDSLALSLRGLPTLISELTRAAHGNTNAEARAQQIYATTLSLVAKSLKAHKEMQNKQILPEEVVLDFSETASSCQGLDIFSENVAVQIHLNGSVSIHL

SEQ ID NO: 23 - DNA, 957 bp, Chlamydia muridarum
atggcatccaagtctcgtcattatcttaaccagccttggtacattatcttattcatctttgttcttagtctggttgctggtacccttctttcttcagtttcctatgttctatctccaatccaaaaacaagctgcagaatttgatcgtaatcagcaaatgttgatggccgcacaaattatttcctatgacaataaattccaaatatatgctgaaggggattggcaacctgctgtctataatacaaaaaaacagatactagaaaaaagctcttccactccaccacaagtgactgtggcgactctatgctcttattttcaaaattttgttagagttttgcttacagactcccaagggaatctttcttcttttgaagatcacaatcttaacctagaagagttcttatcccaccccacatcttcagtacaagatcactctctgcatgtaatttatgctattctagcaaacgatgaatcctctaaaaagttatcatcctcccaagtagcaaaaaatccggtatccatagagtctattattcttcctataaaaggatttggtttatggggaccaatctatggatttcttgctttagaaaaggacggtaatacggttctagggacatgctggtatcaacatggtgagactccaggattaggagcaaatataactaatccccaatggcaacaaaatttcagaggaaaaaaagtatttctcgcttcctcttccggagaaaccgattttgctaaaacaactctaggactagaagttataaaaggatctgtttctgcattattaggggactctcccaaagctaattccgctgttgatggaatttcaggagctacactgacctgtaatggagttactgaagcttttgctaattcgctagctccttaccgccccttattgactttcttcgccaatcttaactctagtggagaatctcatgacaaccaataa

SEQ ID NO: 24 - protein, 318 aa, Chlamydia muridarum
MASKSRHYLNQPWYIILFIFVLSLVAGTLLSSVSYVLSPIQKQAAEFDRNQQMLMAAQIISYDNKFQIYAEGDWQPAVYNTKKQILEKSSSTPPQVTVATLCSYFQNFVRVLLTDSQGNLSSFEDHNLNLEEFLSHPTSSVQDHSLHVIYAILANDESSKKLSSSQVAKNPVSIESIILPIKGFGLWGPIYGFLALEKDGNTVLGTCWYQHGETPGLGANITNPQWQQNFRGKKVFLASSSGETDFAKTTLGLEVIKGSVSALLGDSPKANSAVDGISGATLTCNGVTEAFANSLAPYRPLLTFFANLNSSGESHDNQ

SEQ ID NO: 25 - DNA, 1416 bp, Chlamydia muridarum
atgaatggaaaagttctgtgtgaggtttctgtgtccttccgttcgattctgctgacggctctgctttcactttcttttacaaacactatgcaggctgcacaccatcattatcaccgttatgatgataaactacgcagacaataccataaaaaggacttgcccactcaagagaatgttcggaaagagttttgtaatccctactctcatagtagtgatcctatccctttgtcacaacaacgaggagtcctatctcctatctgtgatttagtctcagagtgctcgtttttgaacgggatttccgttaggagtcttaaacaaacactgaaaaattctgctgggactcaagttgctttagactggtctatccttcctcaatggttcaatcctagatcctcttgggctcctaagctctctattcgagatcttggatatggtaaaccccagtcccttattgaagcagattccccttgttgtcaaacctgcttcaacccatctgctgctattacgatttacgattcttcatgtgggaagggtgttgtccaagtgtcatacacccttgttcgttattggagagaaacggctgcacttgcagggcaaactatgatgcttgcaggaagtattaatgattatcctgctcgccaaaacatattctctcaacttacattttcccaaactttccctaatgagagagtaaatctaactgttggtcaatactctctttactcgatagacggaacgctgtacaacaatgatcagcagctaggatttattagttatgcgttgtcgcaaaatccaacagcgacttattcctctggaagccttggcgcctatctacaagtcgctccaacagaaagcacctgtcttcaagttgggttccaagatgcctataatatttcaggttcctcgatcaaatggaataatcttacaaaaaataagtataacttccatggctatgcatcttgggctccacactgttgcttaggacctggacaatactctgttcttctttatgtaaccagaaaggttcctgagcaaatgatgcagacaatgggctggtctgtgaatgcaagtcaatacatctcttctaaactttatgtatttggaagatacagcggagtcacaggccaattgtctcctattaaccgaacctattcatttggcttagtctctcctaatttattgaaccgtaacccacaagacttatttggagtagcttgcgcattcaataatatacacgcctccgcctttcaaaatgctcaaagaaaatatgaaactgtgatcgagggatttgcaactattggttgcggaccttacatctcctttgctccagatttccaactttacctctatcctgctctgcgtccaaataaacaaagcgcccgagtctatagcgttcgcgcaaacctagctatttag

SEQ ID NO: 26 - protein, 471 aa, Chlamydia muridarum
MNGKVLCEVSVSFRSILLTALLSLSFTNTMQAAHHHYHRYDDKLRRQYHKKDLPTQENVRKEFCNPYSHSSDPIPLSQQRGVLSPICDLVSECSFLNGISVRSLKQTLKNSAGTQVALDWSILPQWFNPRSSWAPKLSIRDLGYGKPQSLIEADSPCCQTCFNPSAAITIYDSSCGKGVVQVSYTLVRYWRETAALAGQTMMLAGSINDYPARQNIFSQLTFSQTFPNERVNLTVGQYSLYSIDGTLYNNDQQLGFISYALSQNPTATYSSGSLGAYLQVAPTESTCLQVGFQDAYNISGSSIKWNNLTKNKYNFHGYASWAPHCCLGPGQYSVLLYVTRKVPEQMMQTMGWSVNASQYISSKLYVFGRYSGVTGQLSPINRTYSFGLVSPNLLNRNPQDLFGVACAFNNIHASAFQNAQRKYETVIEGFATIGCGPYISFAPDFQLYLYPALRPNKQSARVYSVRANLAI

SEQ ID NO: 27 - DNA, 1665 bp, Chlamydia muridarum
atgcgaataggagatcctatgaacaaactcatcagacgagctgtgacgatcttcgcggtgactagtgtggcgagtttatttgctagcggggtgttagagacctctatggcagagtctctctctaccaacgttattagcttagctgacaccaaagcgaaagagaccacttctcatcaaaaagacagaaaagcaagaaaaaatcatcaaaataggacttccgtagtccgtaaagaggttactgcagttcgtgatactaaagctgtagagcctagacaggattcttgctttggcaaaatgtatacagtcaaagttaatgatgatcgtaatgtagaaatcgtgcagtccgttcctgaatatgctacggtaggatctccatatcctattgagattactgctatagggaaaagagactgtgttgatgtaatcattacacagcaattaccatgcgaagcagagtttgttagcagtgatccagctactactcctactgctgatggtaagctagtttggaaaattgatcggttaggacagggcgaaaagagtaaaattactgtatgggtaaaacctcttaaagaaggttgctgctttacagctgcaacggtttgtgcttgtccagagatccgttcggttacgaaatgtggccagcctgctatctgtgttaaacaggaaggtccagaaagcgcatgtttgcgttgcccagtaacttatagaattaatgtagtcaaccaaggaacagcaacagcacgtaatgttgttgtggaaaatcctgttccagatggctatgctcatgcatccggacagcgtgtattgacatatactcttggggatatgcaacctggagaacagagaacaatcaccgtggagttttgtccgcttaaacgtggtcgagtcacaaatattgctacagtttcttactgtggtggacacaaaaatactgctagcgtaacaacagtgatcaatgagccttgcgtgcaagttaacatcgagggagcagattggtcttatgtttgtaagcctgtagaatatgttatctctgtttctaaccctggtgacttagttttacgagacgttgtaattgaagatacgctttctcctggaataactgttgttgaagcagctggagctcagatttcttgtaataaattggtttggactttgaaggaactcaatcctggagagtctttacaatataaggttctagtaagagctcaaactccagggcaattcacaaacaacgttgttgtgaaaagttgctctgattgcggtatttgtacttcttgcgcagaagcaacaacttactggaaaggagttgctgctactcatatgtgcgtagtagatacttgtgatcctatttgcgtaggagagaacactgtttatcgtatctgtgtgacaaacagaggttctgctgaagatacaaatgtgtccttaattttgaaattctctaaagaattacaacctatatctttctctggaccaactaaaggaaccattacaggaaacacggtagtgtttgattcgttacctagattaggttctaaagaaactgtagagttttctgtaacgttgaaagcagtatccgctggagatgctcgtggggaagctattctttcttccgatacattgacagttcctgtatctgatacggagaatacacatatctattaa

SEQ ID NO: 28 - protein, 554 aa, Chlamydia muridarum
MRIGDPMNKLIRRAVTIFAVTSVASLFASGVLETSMAESLSTNVISLADTKAKETTSHQKDRKARKNHQNRTSVVRKEVTAVRDTKAVEPRQDSCFGKMYTVKVNDDRNVEIVQSVPEYATVGSPYPIEITAIGKRDCVDVIITQQLPCEAEFVSSDPATTPTADGKLVWKIDRLGQGEKSKITVWVKPLKEGCCFTAATVCACPEIRSVTKCGQPAICVKQEGPESACLRCPVTYRINVVNQGTATARNVVVENPVPDGYAHASGQRVLTYTLGDMQPGEQRTITVEFCPLKRGRVTNIATVSYCGGHKNTASVTTVINEPCVQVNIEGADWSYVCKPVEYVISVSNPGDLVLRDVVIEDTLSPGITVVEAAGAQISCNKLVWTLKELNPGESLQYKVLVRAQTPGQFTNNVVVKSCSDCGICTSCAEATTYWKGVAATHMCVVDTCDPICVGENTVYRICVTNRGSAEDTNVSLILKFSKELQPISFSGPTKGTITGNTVVFDSLPRLGSKETVEFSVTLKAVSAGDARGEAILSSDTLTVPVSDTENTHIY

SEQ ID NO: 29 - DNA, 504 bp, Chlamydia muridarum
atgtccagacagaatgctgaggaaaatctaaaaaattttgctaaagagctcaagctccccgacgtggccttcgatcagaataatacgtgcattttgtttgttgatggagagttttctcttcacctgacctacgaagagcactctgatcgcctttatgtttacgcacctctccttgacggactcccagataatccgcaaagaaagttggctctgtatgagaaattgttggaaggctctatgctcggaggccaaatggctggtggaggagtaggagttgctactaaagaacagttgatcctaatgcattgcgtgttagatatgaaatatgcagagactaatctattgaaagcttttgcacagcttttcattgaaactgttgtgaaatggcgaacggtctgttctgatatcagcgctggacgagaaccttccgttgacactatgcctcaaatgcctcaaggaggcagcggaggaattcaacctcctccaacaggaattcgtgcgtag

SEQ ID NO: 30 - protein, 167 aa, Chlamydia muridarum
MSRQNAEENLKNFAKELKLPDVAFDQNNTCILFVDGEFSLHLTYEEHSDRLYVYAPLLDGLPDNPQRKLALYEKLLEGSMLGGQMAGGGVGVATKEQLILMHCVLDMKYAETNLLKAFAQLFIETVVKWRTVCSDISAGREPSVDTMPQMPQGGSGGIQPPPTGIRA

SEQ ID NO: 31 - protein, 809 aa, Chlamydia muridarum
MPHSPFLYVVQPHSVFNPRLGERHPITLDFIKEKNRLADFIENLPLEIFGAPSFLENASLEASYVLSRESTKDGTLFTVLEPKLSACVATCLVDSSIPMEPDNELLEEIKHTLLKSSCDGVQYRVTRETLQNKDEAPRVSLVADDIELIRNVDFLGRSVDIVKLDPLNIPNTVSEENALDYSFTRETAKLSPDGRVGIPQGTKILPAPSLEVEISTSIFEETSSFEQNFSSSITFCVPPLTSFSPLQEPPLVGAGQQEILVTKKHLFPSYTPKLIDIVKRHKRDAKILVNKIQFEKLWRSHAKSQILKEGSVRLDLQGFTGELFNYQLQVGSHTIAAVLIDPEIANVKSLPEQTYAVRKIKSGFQCSLDDQHIYQVAVKKHLSLSSQPPKISPLSQSESSDLSLFEAAAFSASLTYEFVKKNTYHAKNTVTCSTVSHSLYILKEDDGANAAEKRLDNSFRNWVENKLNANSPDSCTAFIQKFGTHYITSATFGGSGFQVLKLSFEQVEGLRSKKISLEAAAANSLLKSSVSNSTESGYSTYDSSSSSHTVFLGGTVLPSVHDGQLDFKDWSESVCLEPVPIHISLLPLTDLLTPLYFPETDTTELSNKRNALQQAVRVYLKDHRSAKQSERSVFTAGINSPSSWFTLESANSPLVVSSPYMTYWSTLPYLFPTLKERSSAAPIVFYFCVDNNEHASQKILNQTYCFIGSLPIRQKIFGREFAENPYLSFYGRFGEAYFDGGYPERCGWIVEKLNTTKDQILRDEDEVQLKHVYSGEYLSTIPIKDSHCTLSRTCTESNAVFIIKKPSSY

SEQ ID NO: 32 - DNA, 609 bp, Chlamydia muridarum
atgctcgctaatcggttatttctaatcacccttataggttttggctattctgcttacggtgccagcacagggaaatcaccttctttacaggttattttagctgaagtcgaggatacatcttcgcgcttacaagctcatcagaatgagcttgttatgctctcggaacgtttagatgagcaagacacaaaacttcaacaactctcgtcaactcaggcccgtaatcttcctcaacaagttcaacggcttgagattgatctgagagctctggctaaaacagctgctgtgctctcgcaatctgttcaggatatccgatcatccgtgcaaaataaattacaagaaatccaacaagaacaaaaaaatttagctcaaaatttacgagcgcttcgcaactccttacaagcactagttgatggctcttccccagaaaattatattgattttttggccggggagacacctgaacatattcacgttgttaaacaaggagaaaccctgagtaaaatcgctagtaagtacaatatccctgtcgcagaattgaaaaaacttaataaattaaattccgatactatttttactgatcaaagaatccgacttccaaaaaagaaataa

SEQ ID NO: 33 - protein, 202 aa, Chlamydia muridarum
MLANRLFLITLIGFGYSAYGASTGKSPSLQVILAEVEDTSSRLQAHQNELVMLSERLDEQDTKLQQLSSTQARNLPQQVQRLEIDLRALAKTAAVLSQSVQDIRSSVQNKLQEIQQEQKNLAQNLRALRNSLQALVDGSSPENYIDFLAGETPEHIHVVKQGETLSKIASKYNIPVAELKKLNKLNSDTIFTDQRIRLPKKK

SEQ ID NO: 34 - protein, 259 aa, Chlamydia muridarum
MSMYIKRKKAWMTFLAIVCSFCLAGCSKESKDSVSEKFIVGTNATYPPFEFVDERGETVGFDIDLAREISKKLGKKLEVREFAFDALVLNLKQHRIDAIMAGVSITSSRLKEILMIPYYGEEIKSLVLVFKDGDSKSLPLDQYNSVAVQTGTYQEEYLQSLPGVRIRSFDSTLEVLMEVLHSKSPIAVLEPSIAQVVLKDFPTLTTETIDLPEDKWVLGYGIGVASDRPSLASDIEAAVQEIKKEGVLAELEQKWGLNG

SEQ ID NO: 35 - protein, 1007 aa, Chlamydia muridarum
MTTPISNSPSSIPTVTVSTTTASSGSLGTSTVSSTTTSTSVAQTATTTSSASTSIIQSSGENIQSTTGTPSPITSSVSTSAPSPKASATANKTSSAVSGKITSQETSEESETQATTSDGEVSSNYDDVDTPTNSSDSTVDSDYQDVETQYKTISNNGENTYETIGSHGEKNTHVQESHASGTGNPINNQQEAIRQLRSSTYTTSPRNENIFSPGPEGLPNMSLPSYSPTDKSSLLAFLSNPNTKAKMLEHSGHLVFIDTTRSSFIFVPNGNWDQVCSMKVQNGKTKEDLGLKDLEDMCAKFCTGYNKFSSDWGNRVDPLVSSKAGIESGGHLPSSVIINNKFRTCVAYGPWNPKENGPNYTPSAWRRGHRVDFGKIFDGTAPFNKINWGSSPTPGDDGISFSNETIGSEPFATPPSSPSQTPVINVNVNVGGTNVNIGDTNVSKGSGTPTSSQSVDMSTDTSDLDTSDIDTNNQTNGDINTNDNSNNVDGSLSDVDSRVEDDDGVSDTESTNGNDSGKTTSTEENGDPSGPDILAAVRKHLDTVYPGENGGSTEGPLPANQNLGNVIHDVEQNGSAKETIITPGDTGPTDSSSSVDADADVEDTSDTDSGIGDDDGVSDTESTNGNNSGKTTSTEENGDPSGPDILAAVRKHLDTVYPGENGGSTEGPLPANQNLGNVIHDVEQNGAAQETIITPGDTESTDTSSSVNANADLEDVSDADSGFGDDDGISDTESTNGNDSGKNTPVGDGGTPSGPDILAAVRKHLDTVYPGENGGSTERPLPANQNLGDIIHDVEQNGSAKETVVSPYRGGGGNTSSPIGLASLLPATPSTPLMTTPRTNGKAAASSLMIKGGETQAKLVKNGGNIPGETTLAELLPRLRGHLDKVFTSDGKFTNLNGPQLGAIIDQFRKETGSGGIIAHTDSVPGENGTASPLTGSSGEKVSLYDAAKNVTQALTSVTNKVTLAMQGQKLEGIINNNNTPSSIGQNLFAAARATTQSLSSLIGTVQ

SEQ ID NO: 36 - protein, 15 aa, Chlamydia muridarum
DYFNDEFFNRFFGLP

SEQ ID NO: 37 - protein, 5 aa, Chlamydia muridarum
SHREQ

SEQ ID NO: 38 - protein, 15 aa, Chlamydia muridarum
ALQKMGVRVQNLTPE

SEQ ID NO: 39 - protein, 15 aa, Chlamydia muridarum
NQVLKNAKGENVLLM

SEQ ID NO: 40 - protein, 20 aa, Chlamydia muridarum
SPMLGYSAPKKDSSTGICLA

SEQ ID NO: 41 - protein, 20 aa, Chlamydia muridarum
EDLLKEVSRGFSKVAAQATP

SEQ ID NO: 42 - protein, 20 aa, Chlamydia muridarum
TGSQAIASPGNKRGFQENPF

SEQ ID NO: 43 - protein, 10 aa, Chlamydia muridarum
PRPQQRDAVR

SEQ ID NO: 44 - protein, 30 aa, Chlamydia muridarum
IAIGNPFGLQATVTVGVISAKGRNQLHIVD

SEQ ID NO: 45 - protein, 30 aa, Chlamydia muridarum
NTAIVSGSGGYIGIGFAIPSLMAKRVIDQL

SEQ ID NO: 46 - protein, 17 aa, Chlamydia muridarum
VAAQATPGVVYIENFPK

SEQ ID NO: 47 - protein, 33 aa, Chlamydia muridarum
GFQENPFDYFNDEFFNRFFGLPSHREQPRPQQR

SEQ ID NO: 48 - protein, 24 aa, Chlamydia muridarum
GTGFIVSEDGYVVTNHHVVEDAGK

SEQ ID NO: 49 - protein, 11 aa, Chlamydia muridarum
TDLAVIKIQAK

SEQ ID NO: 50 - protein, 13 aa, Chlamydia muridarum
VIDQLISDGQVTR

SEQ ID NO: 51 - protein, 24 aa, Chlamydia muridarum
AGLRQEDVIVAYNGKEVESLSALR

SEQ ID NO: 52 - protein, 22 aa, Chlamydia muridarum
FIEIPVTVTQIPAEDGVSALQK

SEQ ID NO: 53 - protein, 10 aa, Chlamydia muridarum
VQNLTPEICK

SEQ ID NO: 54 - protein, 18 aa, Chlamydia muridarum
NAKGENVLLMVSQGEVIR

SEQ ID NO: 55 - protein, 15 aa, Chlamydia muridarum
GENVLLMVSQGEVIR

SEQ ID NO: 56 - protein, 15 aa, Chlamydia trachomatis
DYFNDEFFNRFFGLP

SEQ ID NO: 57 - protein, 5 aa, Chlamydia trachomatis
SHREQ

SEQ ID NO: 58 - protein, 15 aa, Chlamydia trachomatis
ALQKMGVRVQNITPE

SEQ ID NO: 59 - protein, 15 aa, Chlamydia trachomatis
NQVLKNSKGENVLLM

SEQ ID NO: 60 - protein, 20 aa, Chlamydia trachomatis
SPMLGYSASKKDSKADICLA

SEQ ID NO: 61 - protein, 20 aa, Chlamydia trachomatis
EDLLKEVSRGFSRVAAKATP

SEQ ID NO: 62 - protein, 20 aa, Chlamydia trachomatis
TGNQAIASPGNKRGFQENPF

SEQ ID NO: 63 - protein, 30 aa, Chlamydia trachomatis; identical to SEQ ID NO: 44

SEQ ID NO: 64 - protein, 30 aa, Chlamydia muridarum; identical to SEQ ID NO: 45

SEQ ID NO: 65 - protein, 6 aa, Artificial Sequence
  protein linker sequence
GSGGGG

SEQ ID NO: 66 - DNA, 26 bp, Artificial Sequence
  immunostimulatory oligonucleotide
  modified_base 1, 3, 5, 7, 9, 11, 13, 15, 17, 19, 21, 23, 25: 'n' is  i
ncncncncncncncncncncncncnc

SEQ ID NO: 67 - protein, 11 aa, Artificial Sequence
  polycationic olipopeptide
KLKLLLLLKLK

SEQ ID NO: 68 - DNA, 20 bp, Artificial Sequence
  primer
tctggaatcgaactctctcg

SEQ ID NO: 69 - DNA, 42 bp, Artificial Sequence
  primer
attttgagacacaacgtggctttcatggcttaccccttgttg

SEQ ID NO: 70 - DNA, 39 bp, Artificial Sequence
  primer
ttcacgaggcagacctcataaacatctgcgtttcccttg

SEQ ID NO: 71 - DNA, 20 bp, Artificial Sequence
  primer
ttgcttctgctttaactcgg

SEQ ID NO: 72 - DNA, 23 bp, Artificial Sequence
  primer
atgagccatattcaacgggaaac

SEQ ID NO: 73 - DNA, 25 bp, Artificial Sequence
  primer
ttagaaaaactcatcgagcatcaaa

SEQ ID NO: 74 - DNA, 18 bp, Artificial Sequence
  primer
cggacccgtattcttaac

SEQ ID NO: 75 - DNA, 18 bp, Artificial Sequence
  primer
gccttcgctttagcatct

SEQ ID NO: 76 - DNA, 19 bp, Artificial Sequence
  primer
gatcggttggttggcagat

SEQ ID NO: 77 - DNA, 43 bp, Artificial Sequence
  primer
caccaggatttatttattctgcgtttttgcgcctcgttatcat

SEQ ID NO: 78 - DNA, 39 bp, Artificial Sequence
  primer
tactgcgatgagtggcaggcgcaggcttaagttctcgtc

SEQ ID NO: 79 - DNA, 20 bp, Artificial Sequence
  primer
aaaatcttgaaagcggttgg

SEQ ID NO: 80 - DNA, 23 bp, Artificial Sequence
  primer
cgcagaataaataaatcctggtg

SEQ ID NO: 81 - DNA, 19 bp, primer
cctgccactcatcgcagta

SEQ ID NO: 82 - DNA, 20 bp, Artificial Sequence
  primer
atgaaaaagacagctatcgc

SEQ ID NO: 83 - DNA, 19 bp, Artificial Sequence
  primer
ttaagcctgcggctgagtt

SEQ ID NO: 84 - protein, 25 aa, Chlamydia muridarum
NKRGFQENPFDYFNDEFFNRFFGLP

SEQ ID NO: 85 - protein, 12 aa, Chlamydia muridarum
TPGVVYIENFPK

SEQ ID NO: 86 - protein, 15 aa, Chlamydia trachomatis
GENVLLMVSQGDVVR